European Patent Application EP 4 470 569 A1, published December 4, 2024. Title: 糖皮质激素的药物偶联物. Applicant: 上海盛迪医药有限公司. The sequence listing filed with the application follows.

SEQUENCE LISTING (52 sequences)

SEQ ID NO: 1 - protein, 118 aa, Artificial Sequence
EVQLVESGGGLVKPGGSLKLSCAASGFTFSDYGMHWVRQAPEKGLEWVAFISSGSSIIYYADIVKGRSTISRDNAKNTLFLQMTSLRSEDTAMYYCTRGNKRGFFDYWGQGTILTVSS

SEQ ID NO: 2 - protein, 108 aa
QIVLTQSPALMSASPGEKVTMTCNASSSVSYMYWYQRKPRSSPKPWIYLTSNLASGVPVRFSGSGSGTSYSLTISSMEAEDAATYYCQQWRSNPPMLTFGSGTKLEVK

SEQ ID NO: 3 - protein, 10 aa, Artificial Sequence
GFTFSDYGMH

SEQ ID NO: 4 - protein, 17 aa, Artificial Sequence
FISSGSSIIYYADIVKG

SEQ ID NO: 5 - protein, 9 aa, Artificial Sequence
GNKRGFFDY

SEQ ID NO: 6 - protein, 10 aa, Artificial Sequence
NASSSVSYMY

SEQ ID NO: 7 - protein, 7 aa, Artificial Sequence
LTSNLAS

SEQ ID NO: 8 - protein, 11 aa, Artificial Sequence
QQWRSNPPMLT

SEQ ID NO: 9 - protein, 125 aa, Artificial Sequence
QVQLQQPGTELLKPGASVSLSCKASGYTFTSYWMHWVKQRPGQGLEWIGLIHPNSDTTKFSENFKTRATLTIDKSSSTAYMKLSSLTSEDSAVYYCAKSKIITTIVARHWYFDVWGTGTTVTVSS

SEQ ID NO: 10 - protein, 111 aa, Artificial Sequence
DIVLTQSPPSLAVSLGQRATISCKASQSVDYGGDSYMNWYQQKLGQPPKVLIYAASNLESGIPARFSGSGSGTDFTLNIHPVEEEDVATYYCQHSNENPPTFGGGTKLEIK

SEQ ID NO: 11 - protein, 10 aa, Artificial Sequence
GYTFTSYWMH

SEQ ID NO: 12 - protein, 17 aa, Artificial Sequence
LIHPNSDTTKFSENFKT

SEQ ID NO: 13 - protein, 16 aa, Artificial Sequence
SKIITTIVARHWYFDV

SEQ ID NO: 14 - protein, 15 aa, Artificial Sequence
KASQSVDYGGDSYMN

SEQ ID NO: 15 - protein, 7 aa, Artificial Sequence
AASNLES

SEQ ID NO: 16 - protein, 9 aa, Artificial Sequence
QHSNENPPT

SEQ ID NO: 17 - protein, 445 aa, Artificial Sequence
EVQLVESGGGLVQPGGSLRLSCAASGFTFSDYGMHWVRQAPGKGLEWVAFISSGSSIIYYADIVKGRSTISRDNAKNSLYLQMNSLRAEDTAVYYCTRGNKRGFFDYWGQGTLVTVSSASTKGPSVFPLAPCSRSTSESTAALGCLVKDYFPEPVTVSWNSGALTSGVHTFPAVLQSSGLYSLSSVVTVPSSSLGTKTYTCNVDHKPSNTKVDKRVESKYGPPCPPCPAPEFLGGPSVFLFPPKPKDTLMISRTPEVTCVVVDVSQEDPEVQFNWYVDGVEVHNAKTKPREEQFNSTYRVVSVLTVLHQDWLNGKEYKCKVSNKGLPSSIEKTISKAKGQPREPQVYTLPPSQEEMTKNQVSLTCLVKGFYPSDIAVEWESNGQPENNYKTTPPVLDSDGSFFLYSRLTVDKSRWQEGNVFSCSVMHEALHNHYTQKSLSLSLGK

SEQ ID NO: 18 - protein, 215 aa, Artificial Sequence
EIVLTQSPATLSLSPGERATLSCNASSSVSYMYWYQQKPGQAPRLLIYLTSNLASGIPARFSGSGSGTDFTLTISSLEPEDFAVYYCQQWRSNPPMLTFGGGTKVEIKRTVAAPSVFIFPPSDEQLKSGTASVVCLLNNFYPREAKVQWKVDNALQSGNSQESVTEQDSKDSTYSLSSTLTLSKADYEKHKVYACEVTHQGLSSPVTKSFNRGEC

SEQ ID NO: 19 - protein, 455 aa, Artificial Sequence
EVQLVQSGAEVKKPGASVKVSCKASGYTFTSYWMHWVRQAPGQGLEWMGLIHPNSDTTKFSENFKTRVTMTIDTSISTAYMELSRLRSDDTAVYYCAKSKIITTIVARHWYFDVWGQGTTVTVSSASTKGPSVFPLAPSSKSTSGGTAALGCLVKDYFPEPVTVSWNSGALTSGVHTFPAVLQSSGLYSLSSVVTVPSSSLGTQTYICNVNHKPSNTKVDKKVEPKSCDKTHTCPPCPAPELLGGPSVFLFPPKPKDTLMISRTPEVTCVVVDVSHEDPEVKFNWYVDGVEVHNAKTKPREEQYNSTYRVVSVLTVLHQDWLNGKEYKCKVSNKALPAPIEKTISKAKGQPREPQVYTLPPSREEMTKNQVSLTCLVKGFYPSDIAVEWESNGQPENNYKTTPPVLDSDGSFFLYSKLTVDKSRWQQGNVFSCSVMHEALHNHYTQKSLSLSPGK

SEQ ID NO: 20 - protein, 218 aa, Artificial Sequence
DIVLTQTPLSLSVTPGQPASISCKASQSVDYGGDSYMNWYLQKPGQPPQLLIYAASNLESGVPDRFSGSGSGTDFTLKISRVEAEDVGVYYCQHSNENPPTFGGGTKVEIKRTVAAPSVFIFPPSDEQLKSGTASVVCLLNNFYPREAKVQWKVDNALQSGNSQESVTEQDSKDSTYSLSSTLTLSKADYEKHKVYACEVTHQGLSSPVTKSFNRGEC

SEQ ID NO: 21 - protein, 98 aa, Artificial Sequence
EVQLVESGGGLVQPGGSLRLSCAASGFTFSSYSMNWVRQAPGKGLEWVSYISSSSSTIYYADSVKGRFTISRDNAKNSLYLQMNSLRAEDTAVYYCAR

SEQ ID NO: 22 - protein, 95 aa, Artificial Sequence
EIVLTQSPATLSLSPGERATLSCRASQSVSSYLAWYQQKPGQAPRLLIYDASNRATGIPARFSGSGSGTDFTLTISSLEPEDFAVYYCQQRSNWP

SEQ ID NO: 23 - protein, 98 aa, Artificial Sequence
QVQLVQSGAEVKKPGASVKVSCKASGYTFTGYYMHWVRQAPGQGLEWMGWINPNSGGTNYAQKFQGRVTMTRDTSISTAYMELSRLRSDDTAVYYCAR

SEQ ID NO: 24 - protein, 100 aa, Artificial Sequence
DIVMTQTPLSLSVTPGQPASISCKSSQSLLHSDGKTYLYWYLQKPGQPPQLLIYEVSNRFSGVPDRFSGSGSGTDFTLKISRVEAEDVGVYYCMQSIQLP

SEQ ID NO: 25 - protein, 118 aa, Artificial Sequence
EVQLVESGGGLVQPGGSLRLSCAASGFTFSDYGMHWVRQAPGKGLEWVAFISSGSSIIYYADIVKGRFTISRDNAKNSLYLQMNSLRAEDTAVYYCARGNKRGFFDYWGQGTLVTVSS

SEQ ID NO: 26 - protein, 118 aa, Artificial Sequence
EVQLVESGGGLVQPGGSLRLSCAASGFTFSDYGMHWVRQAPGKGLEWVAFISSGSSIIYYADIVKGRFTISRDNAKNSLYLQMNSLRAEDTAVYYCTRGNKRGFFDYWGQGTLVTVSS

SEQ ID NO: 27 - protein, 118 aa, Artificial Sequence
EVQLVESGGGLVQPGGSLRLSCAASGFTFSDYGMHWVRQAPGKGLEWVAFISSGSSIIYYADIVKGRSTISRDNAKNSLYLQMNSLRAEDTAVYYCTRGNKRGFFDYWGQGTLVTVSS

SEQ ID NO: 28 - protein, 108 aa, Artificial Sequence
EIVLTQSPATLSLSPGERATLSCNASSSVSYMYWYQQKPGQAPRLLIYLTSNLASGIPARFSGSGSGTDFTLTISSLEPEDFAVYYCQQWRSNPPMLTFGGGTKVEIK

SEQ ID NO: 29 - protein, 108 aa, Artificial Sequence
EIVLTQSPATLSLSPGERATLSCNASSSVSYMYWYQQKPGQAPRLLIYLTSNLASGIPARFSGSGSGTDYTLTISSLEPEDFAVYYCQQWRSNPPMLTFGGGTKVEIK

SEQ ID NO: 30 - protein, 108 aa, Artificial Sequence
EIVLTQSPATLSLSPGERATLSCNASSSVSYMYWYQQKPGQAPRPWIYLTSNLASGIPARFSGSGSGTDYTLTISSLEPEDFAVYYCQQWRSNPPMLTFGGGTKVEIK

SEQ ID NO: 31 - protein, 125 aa, Artificial Sequence
EVQLVQSGAEVKKPGASVKVSCKASGYTFTSYWMHWVRQAPGQGLEWMGLIHPNSDTTKFSENFKTRVTMTRDTSISTAYMELSRLRSDDTAVYYCARSKIITTIVARHWYFDVWGQGTTVTVSS

SEQ ID NO: 32 - protein, 125 aa, Artificial Sequence
EVQLVQSGAEVKKPGASVKVSCKASGYTFTSYWMHWVRQAPGQGLEWMGLIHPNSDTTKFSENFKTRVTMTIDTSISTAYMELSRLRSDDTAVYYCAKSKIITTIVARHWYFDVWGQGTTVTVSS

SEQ ID NO: 33 - protein, 125 aa, Artificial Sequence
EVQLVQSGAEVKKPGASVKVSCKASGYTFTSYWMHWVRQAPGQGLEWMGLIHPNSDTTKFSENFKTRVTLTIDKSISTAYMELSRLRSDDTAVYYCAKSKIITTIVARHWYFDVWGQGTTVTVSS

SEQ ID NO: 34 - protein, 111 aa, Artificial Sequence
DIVMTQTPLSLSVTPGQPASISCKASQSVDYGGDSYMNWYLQKPGQPPQLLIYAASNLESGVPDRFSGSGSGTDFTLKISRVEAEDVGVYYCQHSNENPPTFGGGTKVEIK

SEQ ID NO: 35 - protein, 111 aa, Artificial Sequence
DIVLTQTPLSLSVTPGQPASISCKASQSVDYGGDSYMNWYLQKPGQPPQLLIYAASNLESGVPDRFSGSGSGTDFTLKISRVEAEDVGVYYCQHSNENPPTFGGGTKVEIK

SEQ ID NO: 36 - protein, 111 aa, Artificial Sequence
DIVMTQTPLSLSVTPGQPASISCKASQSVDYGGDSYMNWYLQKPGQPPQLLIYAASNLESGIPDRFSGSGSGTDFTLKISRVEAEDVGVYYCQHSNENPPTFGGGTKVEIK

SEQ ID NO: 37 - protein, 108 aa, Artificial Sequence
EIVLTQSPATLSLSPGERATLSCRASSSVPYMYWYQQKPGQAPRLLIYLTSNLASGIPARFSGSGSGTDFTLTISSLEPEDFAVYYCQQWRAYPPMLTFGGGTKVEIK

SEQ ID NO: 38 - protein, 10 aa, Artificial Sequence
RASSSVPYMY

SEQ ID NO: 39 - protein, 7 aa, Artificial Sequence
LASSRPS

SEQ ID NO: 40 - protein, 11 aa, Artificial Sequence
QQWRAYPPMLT

SEQ ID NO: 41 - protein, 108 aa, Artificial Sequence
EIVLTQSPATLSLSPGERATLSCRASPGVPPLAWYQQKPGQAPRLLIYLASSRPSGIPARFSGSGSGTDFTLTISSLEPEDFAVYYCQQWRSNPPMLTFGGGTKVEIK

SEQ ID NO: 42 - protein, 10 aa, Artificial Sequence
RASPGVPPLA

SEQ ID NO: 43 - protein, 118 aa, Artificial Sequence
EVQLVESGGGLVQPGGSLRLSCAASGFTFSDYGMHWVRQAPGKGLEWVAFISSGSSIIYYADIVKGRSTISRDNAKNTLYLQMNSLRAEDTAVYYCTRGNKRGFFDYWGQGTLVTVSS

SEQ ID NO: 44 - protein, 445 aa, Artificial Sequence
EVQLVESGGGLVQPGGSLRLSCAASGFTFSDYGMHWVRQAPGKGLEWVAFISSGSSIIYYADIVKGRSTISRDNAKNTLYLQMNSLRAEDTAVYYCTRGNKRGFFDYWGQGTLVTVSSASTKGPSVFPLAPCSRSTSESTAALGCLVKDYFPEPVTVSWNSGALTSGVHTFPAVLQSSGLYSLSSVVTVPSSSLGTKTYTCNVDHKPSNTKVDKRVESKYGPPCPPCPAPEFLGGPSVFLFPPKPKDTLMISRTPEVTCVVVDVSQEDPEVQFNWYVDGVEVHNAKTKPREEQFNSTYRVVSVLTVLHQDWLNGKEYKCKVSNKGLPSSIEKTISKAKGQPREPQVYTLPPSQEEMTKNQVSLTCLVKGFYPSDIAVEWESNGQPENNYKTTPPVLDSDGSFFLYSRLTVDKSRWQEGNVFSCSVMHEALHNHYTQKSLSLSLGK

SEQ ID NO: 45 - protein, 215 aa, Artificial Sequence
EIVLTQSPATLSLSPGERATLSCRASSSVPYMYWYQQKPGQAPRLLIYLTSNLASGIPARFSGSGSGTDFTLTISSLEPEDFAVYYCQQWRAYPPMLTFGGGTKVEIKRTVAAPSVFIFPPSDEQLKSGTASVVCLLNNFYPREAKVQWKVDNALQSGNSQESVTEQDSKDSTYSLSSTLTLSKADYEKHKVYACEVTHQGLSSPVTKSFNRGEC

SEQ ID NO: 46 - protein, 215 aa, Artificial Sequence
EIVLTQSPATLSLSPGERATLSCRASPGVPPLAWYQQKPGQAPRLLIYLASSRPSGIPARFSGSGSGTDFTLTISSLEPEDFAVYYCQQWRSNPPMLTFGGGTKVEIKRTVAAPSVFIFPPSDEQLKSGTASVVCLLNNFYPREAKVQWKVDNALQSGNSQESVTEQDSKDSTYSLSSTLTLSKADYEKHKVYACEVTHQGLSSPVTKSFNRGEC

SEQ ID NO: 47 - protein, 448 aa, Artificial Sequence
EVQLVESGGGLVQPGGSLRLSCAASGFTFSDYGMHWVRQAPGKGLEWVAFISSGSSIIYYADIVKGRSTISRDNAKNTLYLQMNSLRAEDTAVYYCTRGNKRGFFDYWGQGTLVTVSSASTKGPSVFPLAPSSKSTSGGTAALGCLVKDYFPEPVTVSWNSGALTSGVHTFPAVLQSSGLYSLSSVVTVPSSSLGTQTYICNVNHKPSNTKVDKKVEPKSCDKTHTCPPCPAPELLGGPSVFLFPPKPKDTLMISRTPEVTCVVVDVSHEDPEVKFNWYVDGVEVHNAKTKPREEQYNSTYRVVSVLTVLHQDWLNGKEYKCKVSNKALPAPIEKTISKAKGQPREPQVYTLPPSRDELTKNQVSLTCLVKGFYPSDIAVEWESNGQPENNYKTTPPVLDSDGSFFLYSKLTVDKSRWQQGNVFSCSVMHEALHNHYTQKSLSLSPGK

SEQ ID NO: 48 - protein, 216 aa, Artificial Sequence
EVQLVESGGGLVQPGGSLRLSCAASGFTFSDYGMHWVRQAPGKGLEWVAFISSGSSIIYYADIVKGRSTISRDNAKNSLYLQMNSLRAEDTAVYYCTRGNKRGFFDYWGQGTLVTVSSASTKGPSVFPLAPCSRSTSESTAALGCLVKDYFPEPVTVSWNSGALTSGVHTFPAVLQSSGLYSLSSVVTVPSSSLGTKTYTCNVDHKPSNTKVDKRV

SEQ ID NO: 49 - protein, 216 aa, Artificial Sequence
EVQLVESGGGLVQPGGSLRLSCAASGFTFSDYGMHWVRQAPGKGLEWVAFISSGSSIIYYADIVKGRSTISRDNAKNSLYLQMNSLRAEDTAVYYCTRGNKRGFFDYWGQGTLVTVSSASTKGPSVFPLAPSSKSTSGGTAALGCLVKDYFPEPVTVSWNSGALTSGVHTFPAVLQSSGLYSLSSVVTVPSSSLGTQTYICNVNHKPSNTKVDKKV

SEQ ID NO: 50 - protein, 216 aa, Artificial Sequence
EVQLVESGGGLVQPGGSLRLSCAASGFTFSDYGMHWVRQAPGKGLEWVAFISSGSSIIYYADIVKGRSTISRDNAKNTLYLQMNSLRAEDTAVYYCTRGNKRGFFDYWGQGTLVTVSSASTKGPSVFPLAPCSRSTSESTAALGCLVKDYFPEPVTVSWNSGALTSGVHTFPAVLQSSGLYSLSSVVTVPSSSLGTKTYTCNVDHKPSNTKVDKRV

SEQ ID NO: 51 - protein, 216 aa, Artificial Sequence
EVQLVESGGGLVQPGGSLRLSCAASGFTFSDYGMHWVRQAPGKGLEWVAFISSGSSIIYYADIVKGRSTISRDNAKNTLYLQMNSLRAEDTAVYYCTRGNKRGFFDYWGQGTLVTVSSASTKGPSVFPLAPSSKSTSGGTAALGCLVKDYFPEPVTVSWNSGALTSGVHTFPAVLQSSGLYSLSSVVTVPSSSLGTQTYICNVNHKPSNTKVDKKV

SEQ ID NO: 52 - protein, 160 aa, Artificial Sequence
ASDEEIQDVSGTWYLKAMTVDSRCPRAVYNSVTPMTLTTLEGGNLEAKFTAQRKGRWQKYKLVLEKTDEPGKYTASGGRHVAYIIRSHVKDHYIFHSEGLCPGQPVPGVWLVGRDPKNNLEALEDFEKAAGARGLSTESILIPRQSETSSPGSDHHHHHH